European Patent Application EP 4 509 612 A1, published February 19, 2025. Title: 一种S-乳酰谷胱甘肽的制备方法. Applicant: 元素驱动（杭州）生物科技有限公司. Application CN. The sequence listing filed with the application follows.

SEQUENCE LISTING (7 sequences)

SEQ ID NO: 1 - DNA, 2265 bp, Streptococcus thermophilus
  source 1..2265: mol_type = other DNA
atgacattaaaccaacttcttcaaaaactggaagctaccagccctattctccaagctaattttggaatcgagcgcgagagtctacgtgtcgataggcaaggacaactggtgcatacacctcacccatcctgtctaggagctcgtagtttccacccctatattcagactgatttttgcgagtttcagatggaactcatcacaccagttgccaaatctactactgaggctcgccgatttctgggagctattactgatgtagcaggccgctctattgctacagacgaggttctctggcctttgtccatgccacctcgtctaaaggcagaggagattcaagttgctcaactggaaaatgacttcgaacgccattatcgtaactatttggctgaaaaatacggaactaaactacaagctatctcaggtatccactataatatggaactgggtaaagatttagttgaggccttgttccaagaaagtgatcagaccgatatgattgccttcaaaaacgccctctatcttaagctggctcagaactacttgcgctaccgttgggtgattacctatctctttggggcctcacccatcgccgaacaaggtttctttgaccaggaagttccagaacctgtgcgttccttccgtaacagtgaccacggctatgtcaataaggaagagattcaagtatcctttgtaagtctagaagattatgtctcagccattgaaacctatatcgaacaaggagatttgaatgcagagaaagaattttactcagctgttcgtttccgtggacaaaaggttaatcgttccttccttgacaaaggaatcacctacctagagttccgtaatttcgaccttaacccttttgagcgtatcggtattagtcagactactatggacactgtgcacttactcattttagccttcctttggcttgatagccctgaaaatgtcgaccaagctcttgcacaaggccacgcgttaaatgagaaaattgccctctctcatcctctaaaacctctaccttcggaggctaaaactcaggacattgtaactgccctagaccaactggtgcaacactttggacttggtgactatcatcaagatctggttaaacaagttaaggcagcctttgcggatccaaatcaaacgctctctgcccagctcttaccctatatcaaagacaaatctctagccgaatttgctttaaacaaggctcttgcctatcatgattacgactggactgcccactatgctctcaagggctatgaagagatggaactctccacccagatgttgctctttgatgccatccaaaagggaattcactttgaaatattggatgagcaagatcaattcctaaaactttggcaccaagaccatgttgaatacgtcaaaaacggtaacatgacctcaaaagacaactacgtggttccccttgctatggctaataagaccgtaaccaagaagattctagcagatgctggcttttcagttccttcaggagacgaatttaccagtcttgaggaaggacttgcctactaccctcttatcaaggataagcaaattgttgtcaaacccaagtcaactaactttggtctgggaatttccattttccaagaacctgccagtcttgacaactatcaaaaagcccttgaaattgctttcgcagaagatacctctgtccttgttgaagaatttattccaggaaccgaataccgtttcttcatcttggatgggcgttgtgaggctgtgcttctgcgtgtcgctgccaatgttattggtgatggcaaacacaccattcgtgaactagtcgctcagaaaaatgctaatccattgcgtggccgtgatcaccggtcacctctggaaatcattgagctaggagacatcgaacaactaatgttagctcaacagggttatacacctgatgatattctcccagaaggaaaaaaggtcaatctgcgtcgtaattccaacatctctacaggtggtgactctattgatgtcactgagaccatggattcctcttaccaagaattagccgcagccatggcaactagcatgggcgcctgggcttgcggggttgatctgataattccagatgaaactcaaattgccaccaaggaaaatcctcattgcacctgcattgagctcaactttaacccttcgatgtatatgcacacctactgtgctgagggtcctggccaagctatcactactaaaatcctagataaactttttccagaaatagtggctggtcaaacttaa

SEQ ID NO: 2 - DNA, 408 bp, Escherichia coli
  source 1..408: mol_type = other DNA
atgcgtcttcttcataccatgctgcgcgttggcgatttgcaacgctccatcgatttttataccaaagtgctgggcatgaaactgctgcgtaccagcgaaaacccggaatacaaatactcactggcgtttgttggctacggcccggaaaccgaagaagcggtgattgaactgacctacaactggggcgtggataaatacgaactcggcactgcttatggtcacatcgcgcttagcgtagataacgccgctgaagcgtgcgaaaaaatccgtcaaaacgggggtaacgtgacccgtgaagcgggtccggtaaaaggcggtactacggttatcgcgtttgtggaagatccggacggttacaaaattgagttaatcgaagagaaagacgccggtcgcggtctgggcaactaa

SEQ ID NO: 3 - DNA, 1417 bp, Escherichia coli
  source 1..1417: mol_type = other DNA
aatggaaaactttaaacatctccctgaaccgttccgcattcgtgttattgagccagtaaaacgtaccactcgcgcttatcgtgaagaggcaattattaaatccggtatgaacccgttcctgctggatagcgaagatgtttttatcgatttactgaccgacagcggcaccggggcggtgacgcagagcatgcaggctgcgatgatgcgcggcgacgaagcctacagcggcagtcgtagctactatgcgttagccgagtcagtgaaaaatatctttggttatcaatacaccattccgactcaccagggccgtggcgcagagcaaatctatattccggtactgattaaaaaacgcgagcaggaaaaaggcctggatcgcagcaaaatggtggcgttctctaactatttctttgataccacgcagggccatagccagatcaacggctgtaccgtgcgtaacgtctatatcaaagaagccttcgatacgggcgtgcgttacgactttaaaggcaactttgaccttgagggattagaacgcggtattgaagaagttggtccgaataacgtgccgtatatcgttgcaaccatcaccagtaactctgcaggtggtcagccggtttcactggcaaacttaaaagcgatgtacagcatcgcgaagaaatacgatattccggtggtaatggactccgcgcgctttgctgaaaacgcctatttcatcaagcagcgtgaagcagaatacaaagactggaccatcgagcagatcacccgcgaaacctacaaatatgccgatatgctggcgatgtccgccaagaaagatgcgatggtgccgatgggcggcctgctgtgcatgaaagacgacagcttctttgatgtgtacaccgagtgcagaaccctttgcgtggtgcaggaaggcttcccgacatatggcggcctggaaggcggcgcgatggagcgtctggcggtaggtctgtatgacggcatgaatctcgactggctggcttatcgtatcgcgcaggtacagtatctggtcgatggtctggaagagattggcgttgtctgccagcaggcgggcggtcacgcggcattcgttgatgccggtaaactgttgccgcatatcccggcagaccagttcccggcacaggcgctggcctgcgagctgtataaagtcgccggtatccgtgcggtagaaattggctctttcctgttaggccgcgatccgaaaaccggtaaacaactgccatgcccggctgaactgctgcgtttaaccattccgcgcgcaacatatactcaaacacatatggacttcattattgaagcctttaaacatgtgaaagagaacgcggcgaatattaaaggattaacctttacgtacgaaccgaaagtattgcgtcacttcaccgcaaaacttaaagaagtttaa

SEQ ID NO: 4 - DNA, 1743 bp, Escherichia coli
  source 1..1743: mol_type = other DNA
atgataaaaccgacgtttttacgccgggtggccattgctgctctgctctcaggaagttgttttagcgccgccgccgcgcctcctgcgccgcccgtctcgtatggtgtggaggaagatgtcttccacccggtacgcgcgaaacagggaatggtagcgtctgtggacgccactgccactcaggtgggggtggatattctcaaggagggcgggaatgccgttgatgccgccgtggcggtgggctacgcgctggcggtaacgcatccgcaggcagggaatctgggcggtggtggttttatgttaatccgctcgaaaaatggcaataccacggctatcgatttccgcgaaatggcacccgccaaagcgacccgcgatatgttcctcgatgatcagggcaacccggacagcaaaaaatcactcacttcgcatctggcttccggcacaccgggtacggtagcaggtttctcgctggcgctggataaatacggcaccatgccgctgaacaaagtcgtgcagcccgcgtttaaactggcacgcgatggttttatcgttaacgacgcgctggctgacgatctcaaaacctacggtagcgaagtgttgccgaatcacgaaaacagtaaagctatcttctggaaagagggcgagccgctgaaaaagggcgacacgctggtgcaggcgaacctggcaaagagcctggagatgattgctgaaaacggcccggacgaattctataaaggcacgattgcggaacagatcgcccaggagatgcagaaaaacggtggcttgatcactaaagaagatttagcagcctataaagcggtcgaacgcactccgataagcggcgattatcgcgggtatcaggtttactccatgccaccgccatcctccggcgggatccatatcgtacaaatcctcaatattctggaaaacttcgatatgaagaaatacggctttggcagcgccgatgcgatgcaaatcatggcagaagcggagaaatacgcctacgccgaccgctcggaatatcttggcgacccggattttgtcaaagtaccgtggcaggcgctgaccaataaagcctatgccaaatctattgccgatcaaattgatatcaataaagcgaagccatccagcgaaattcgccccggcaagcttgcgccttatgagagtaatcaaactacccattactcagtggtggataaagatggtaacgcggtggcggtgacctatacgctgaacaccaccttcggtacgggcattgtcgcgggcgagagcggtattctgcttaataaccagatggatgatttctccgccaaaccgggcgtaccgaacgtttacgggctggtgggcggtgatgccaacgccgtcgggccgaacaaacgcccgctgtcgtcgatgtcgccgaccattgtggtgaaagacggtaaaacctggctggttaccggtagcccaggcggtagccggatcatcactacagtgctgcaaatggtggtgaatagcatcgattatggcttgaacgtcgccgaagcgaccaatgcgccgcgtttccaccatcagtggttgccggacgagctgcgtgtcgaaaaagggtttagcccggatacgctcaagctgctggaagcaaaaggtcagaaagtggcgctgaaagaggcgatgggcagtacacaaagcattatggttgggccggacggtgagttgtacggcgcatccgacccgcgctcggtggatgatttaacggcggggtactaa

SEQ ID NO: 5 - DNA, 756 bp, Escherichia coli
  source 1..756: mol_type = other DNA
atgaatcttaacagtattcccgcctttgatgacaattacatctgggttttgaatgatgaagcaggtcgctgcctgattgtcgatcccggagacgcagagccagtattaaacgccattgccgccaataactggcaaccggaggccatatttctcacccaccatcaccacgatcacgttggcggcgtaaaagaactggtggaaaagtttccacaaattgtggtgtatggtccacaagagacacaagataagggaacaacacaggtagtcaaagatggcgaaactgccttcgttttggggcatgaatttagtgtaattgctacgccgggtcacactttaggacatatctgttacttcagtaaaccttatctattttgcggcgacacactgttttctggtgggtgtggtcggttgtttgaagggacagcatcacaaatgtatcaatcacttaaaaagttaagtgcgttacctgacgatacattggtatgttgtgctcatgaatataccttatcaaatatgaagtttgctttgagtattcttccgcacgatttgtccataaatgattattatcgtaaagttaaggagttacgggcaaaaaatcaaataacactacccgtaattctgaaaaatgagcggcaaattaatgtttttttaagaacggaagatattgatttaattaatgtaattaatgaagaaacattattgcaacaacctgaagagcgttttgcatggttaaggtcaaagaaagataggttctga

SEQ ID NO: 6 - DNA, 648 bp, Escherichia coli
  source 1..648: mol_type = other DNA
atgaactatcgtattattccggtcaccgcattctcccagaactgttcattaatctggtgtgaacaaacccgtctggccgcactggtcgatcctggcggcgatgcggaaaaaatcaaacaggaagttgatgacagcggcctgacactgatgcagatcctgctgacgcatggtcatctggaccacgttggcgcagcggcggaactggcgcaacattacggcgtgccggttttcggcccggaaaaagaagatgagttctggctgcaaggcttgcctgcgcaaagtcgtatgtttggtctggaagagtgccagccgctgacgccagatcgttggctgaacgaaggcgataccatcagcatagggaatgtgactttacaggtgttacattgccctgggcatacgccgggtcatgtcgtgttttttgatgatcgggcaaagctgctgatttctggcgatgttattttcaaaggcggagtagggcgcagtgacttcccgcgtggcgatcataatcaactgatttcttcaatcaaagataaattgctgccactgggggatgacgtgatatttattccgggtcacggaccattatccacacttggttatgaacgcctgcataatcccttcctgcaagacgaaatgcccgtctggtaa

SEQ ID NO: 7 - DNA, 837 bp, Escherichia coli
  source 1..837: mol_type = other DNA
atggaaatgctcgaagagcaccgctgttttgaaggctggcagcaacgctggcgacacgactccagtaccttaaactgcccgatgacgttcagtatctttctccctccacctcgtgatcacactccgccaccagtgctgtactggctttccggattaacctgcaatgacgagaacttcaccaccaaggcgggtgcccagcgggtagcggcggaactggggattgtactggtgatgccagacaccagcccgcgcggcgaaaaggttgccaacgacgatggctacgatttaggccagggcgcaggcttttatcttaatgccacgcaaccgccgtgggcgacgcattaccggatgtatgattatctgcgcgatgaattaccggcgctggttcagtcgcaatttaatgtcagcgaccgctgcgccattagcggtcactcaatgggtggtcacggtgcgctgattatggcgctgaaaaatccgggtaaatacaccagcgtttcggcctttgcgccaattgtgaatccgtgcagcgtcccgtggggaatcaaagcgtttagcagctatttaggtgaggacaaaaatgcatggctggaatgggacagttgcgcactgatgtatgccagtaacgcgcaggatgcgatcccgacgcttatcgatcagggcgataatgatcagtttcttgccgaccagttgcaacctgcggtactggcagaagccgcgcgccagaaagcgtggccgatgacgctgcgtattcagccgggatatgatcacagttactacttcatcgcctcttttatagaggatcacctgcgcttccatgcgcagtatttactgaagtga